European Patent Application EP 4 362 030 A2, published May 1, 2024. Title: BIOINFORMATICS SYSTEMS, APPARATUSES, AND METHODS FOR PERFORMING SECONDARY AND/OR TERTIARY PROCESSING. Applicant: ILLUMINA, INC. Application EP. The sequence listing filed with the application follows.

SEQUENCE LISTING (4 sequences)

SEQ ID NO: 1 - DNA, 11 bp, synthetic construct
  misc_feature 1..11: note = synthetic candidate haplotype
  source 1..11: mol_type = other DNA
cgattctaagt

SEQ ID NO: 2 - DNA, 11 bp, synthetic construct
  misc_feature 1..11: note = synthetic candidate haplotype
  source 1..11: mol_type = other DNA
cgattgtaagt

SEQ ID NO: 3 - DNA, 12 bp, synthetic construct
  misc_feature 1..12: note = synthetic candidate haplotype
  source 1..12: mol_type = other DNA
catgcacatgca

SEQ ID NO: 4 - DNA, 12 bp, synthetic construct
  misc_feature 1..12: note = synthetic candidate haplotype
  source 1..12: mol_type = other DNA
catgcacctgca